European Patent Application EP 4 736 880 A1, published May 6, 2026. Title: NUCLEIC ACID DELIVERY COMPOSITION AND NUCLEIC ACID-CONTAINING COMPOSITION. Applicant: TOKUSHIMA UNIVERSITY. The sequence listing filed with the application follows.

SEQUENCE LISTING (12 sequences)

SEQ ID NO: 1 - protein, 10 aa, synthetic construct
  LIPID <1: note = peptide modified by N-terminal stearoylation
CHHRRRRHHC

SEQ ID NO: 2 - protein, 10 aa, synthetic construct
CHHRRRRHHC

SEQ ID NO: 3 - DNA, 21 bp, synthetic construct
  misc_feature 1..19: note = RNA
  misc_feature 20..21: note = DNA
  source 1..21: mol_type = other DNA; note = sense strand of siRNA
atccgcgcgatagtacgtatt

SEQ ID NO: 4 - DNA, 21 bp, synthetic construct
  misc_feature 1..19: note = RNA
  misc_feature 20..21: note = DNA
  source 1..21: mol_type = other DNA; note = antisense strand of siRNA
tacgtactatcgcgcggattt

SEQ ID NO: 5 - DNA, 20 bp, synthetic construct
  source 1..20: mol_type = other DNA
gttaccagcccaaacctcaa

SEQ ID NO: 6 - DNA, 20 bp, synthetic construct
  source 1..20: mol_type = other DNA
cgatgtggcagagaaatcac

SEQ ID NO: 7 - DNA, 24 bp, synthetic construct
  source 1..24: mol_type = other DNA
tcaacagcaactcccactcttcca

SEQ ID NO: 8 - DNA, 24 bp, synthetic construct
  source 1..24: mol_type = other DNA
accctgttgctgtagccgtattca

SEQ ID NO: 9 - DNA, 16 bp, synthetic construct
  source 1..16: mol_type = other DNA
  modified_base 1..3: mod_base = OTHER; note = LNA
  modified_base 14..16: mod_base = OTHER; note = LNA
  modified_base 1..16: mod_base = OTHER; note = phosphorothioate modification
ctagttcactgaatgc

SEQ ID NO: 10 - DNA, 20 bp, synthetic construct
  source 1..20: mol_type = other DNA
  modified_base 1: mod_base = OTHER; note = 2'-O-methoxyethylcytidine; note = phosphorothioate modification
  modified_base 2: mod_base = OTHER; note = 2'-O-methoxyethyladenosine
  modified_base 3: mod_base = OTHER; note = 2'-O-methoxyethylguanosine; note = phosphorothioate modification
  modified_base 5: mod_base = OTHER; note = phosphorothioate modification; note = 2'-O-methoxyethyladenosine
  modified_base 16: mod_base = OTHER; note = 2'-O-methoxyethylcytidine
  modified_base 17: mod_base = OTHER; note = 2'-O-methoxyethladenosine; note = phosphorothioate modification
  modified_base 18: mod_base = OTHER; note = 2'-O-methoxyethylguanosine
  modified_base 19: mod_base = OTHER; note = 2'-O-methoxyethylcytidine; note = phosphorothioate modification
  modified_base 20: mod_base = OTHER; note = 2'-O-methoxyethyl-5-methyluridine; note = phosphorothioate modification
  modified_base 4: mod_base = OTHER; note = 2'-O-methoxyethylguanosine
  modified_base 6..15: mod_base = OTHER; note = phosphorothioate modification
caggatacatttctacagct

SEQ ID NO: 11 - DNA, 21 bp, synthetic construct
  source 1..21: mol_type = other DNA
catcagccctaatccatctga

SEQ ID NO: 12 - DNA, 21 bp, synthetic construct
  source 1..21: mol_type = other DNA
cgcgactaacaatcaaagtga